European Patent Application EP 4 130 040 A1, published February 8, 2023. Title: Fully Human Anti-human CD22 Chimeric Antigen Receptor and Application Thereof. Applicant: Nanjing IASO Biotherapeutics Co., Ltd. The sequence listing filed with the application follows.

SEQUENCE LISTING (45 sequences)

SEQ ID NO: 1 - protein, 11 aa, Artificial
  Clone 17 LCDR1 amino acid sequence
RASQSISSWLA

SEQ ID NO: 2 - protein, 7 aa, Artificial
  Clone 17 LCDR2 amino acid sequence
KASSLES

SEQ ID NO: 3 - protein, 9 aa, Artificial
  Clone 17 LCDR3 amino acid sequence
QQYERFPWT

SEQ ID NO: 4 - protein, 9 aa, Artificial
  Clone 17 HCDR1 amino acid sequence
FTFSSYAMS

SEQ ID NO: 5 - protein, 17 aa, Artificial
  Clone 17 HCDR2 amino acid sequence
AISGSGGSTYYADSVKG

SEQ ID NO: 6 - protein, 13 aa, Artificial
  Clone 17 HCDR3 amino acid sequence
AKVGISSLHGMDV

SEQ ID NO: 7 - protein, 11 aa, Artificial
  Clone 28 LCDR1 amino acid sequence
RASQSISSWLA

SEQ ID NO: 8 - protein, 7 aa, Artificial
  Clone 28 LCDR2 amino acid sequence
DASSLES

SEQ ID NO: 9 - protein, 9 aa, Artificial
  Clone  28 LCDR3 amino acid sequence
QQANTYSPT

SEQ ID NO: 10 - protein, 9 aa, Artificial
  Clone 28 HCDR1 amino acid sequence
GSISSYYWS

SEQ ID NO: 11 - protein, 16 aa, Artificial
  Clone 28 HCDR2 amino acid sequence
RIYTSGSTNYNPSLKS

SEQ ID NO: 12 - protein, 11 aa, Artificial
  Clone 28 HCDR3 amino acid sequence
ARDLYRDGMDV

SEQ ID NO: 13 - protein, 12 aa, Artificial
  Clone 80 LCDR1 amino acid sequence
RASQSVSSSYLA

SEQ ID NO: 14 - protein, 7 aa, Artificial
  Clone 80 LCDR2 amino acid sequence
GASSRAT

SEQ ID NO: 15 - protein, 9 aa, Artificial
  Clone 80 LCDR3 amino acid sequence
QQAGLFPYT

SEQ ID NO: 16 - protein, 10 aa, Artificial
  Clone 80 HCDR1 amino acid sequence
GSISSSNWWS

SEQ ID NO: 17 - protein, 16 aa, Artificial
  Clone 80 HCDR2 amino acid sequence
EIYHSGSTNYNPSLKS

SEQ ID NO: 18 - protein, 12 aa, Artificial
  Clone 80 HCDR3 amino acid sequence
ARLPGYESAFDI

SEQ ID NO: 19 - protein, 107 aa, Artificial
  Clone 17 VL amino acid sequence
DIQMTQSPSTLSASVGDRVTITCRASQSISSWLAWYQQKPGKAPKLLIYKASSLESGVPSRFSGSGSGTEFTLTISSLQPDDFATYYCQQYERFPWTFGGGTKVEIK

SEQ ID NO: 20 - protein, 120 aa, Artificial
  Clone 17 VH amino acid sequence
EVQLLESGGGLVQPGGSLRLSCAASGFTFSSYAMSWVRQAPGKGLEWVSAISGSGGSTYYADSVKGRFTISRDNSKNTLYLQMNSLRAEDTAVYYCAKVGISSLHGMDVWGQGTTVTVSS

SEQ ID NO: 21 - protein, 107 aa, Artificial
  Clone 28 VL amino acid sequence
DIQMTQSPSTLSASVGDRVTITCRASQSISSWLAWYQQKPGKAPKLLISDASSLESGVPSRFSGSGSGTEFTLTISSLQPDDFATYYCQQANTYSPTFGGGTKVEIK

SEQ ID NO: 22 - protein, 117 aa, Artificial
  Clone 28 VH amino acid sequence
QVQLQESGPGLVKPSETLSLTCTVSGGSISSYYWSWIRQPAGKGLEWIGRIYTSGSTNYNPSLKSRVTMSVDTSKNQFSLKLSSVTAADTAVYYCARDLYRDGMDVWGQGTTVTVSS

SEQ ID NO: 23 - protein, 108 aa, Artificial
  Clone 80 VL amino acid sequence
EIVLTQSPGTLSLSPGERATLSCRASQSVSSSYLAWYQQKPGQAPRLLIYGASSRATGIPDRFSGSGSGTDFTLTISRLEPEDFAVYYCQQAGLFPYTFGGGTKVEIK

SEQ ID NO: 24 - protein, 119 aa, Artificial
  Clone 80 VH amino acid sequence
QVQLQESGPGLVKPSGTLSLTCAVSGGSISSSNWWSWVRQPPGKGLEWIGEIYHSGSTNYNPSLKSRVTISVDKSKNQFSLKLSSVTAADTAVYYCARLPGYESAFDIWGQGTMVTVSS

SEQ ID NO: 25 - protein, 242 aa, Artificial
  Clone 17 scFv amino acid sequence
EVQLLESGGGLVQPGGSLRLSCAASGFTFSSYAMSWVRQAPGKGLEWVSAISGSGGSTYYADSVKGRFTISRDNSKNTLYLQMNSLRAEDTAVYYCAKVGISSLHGMDVWGQGTTVTVSSGGGGSGGGGSGGGGSDIQMTQSPSTLSASVGDRVTITCRASQSISSWLAWYQQKPGKAPKLLIYKASSLESGVPSRFSGSGSGTEFTLTISSLQPDDFATYYCQQYERFPWTFGGGTKVEIK

SEQ ID NO: 26 - protein, 239 aa, Artificial
  Clone 28 scFv amino acid sequence
QVQLQESGPGLVKPSETLSLTCTVSGGSISSYYWSWIRQPAGKGLEWIGRIYTSGSTNYNPSLKSRVTMSVDTSKNQFSLKLSSVTAADTAVYYCARDLYRDGMDVWGQGTTVTVSSGGGGSGGGGSGGGGSDIQMTQSPSTLSASVGDRVTITCRASQSISSWLAWYQQKPGKAPKLLISDASSLESGVPSRFSGSGSGTEFTLTISSLQPDDFATYYCQQANTYSPTFGGGTKVEIK

SEQ ID NO: 27 - protein, 242 aa, Artificial
  Clone 80 scFv amino acid sequence
QVQLQESGPGLVKPSGTLSLTCAVSGGSISSSNWWSWVRQPPGKGLEWIGEIYHSGSTNYNPSLKSRVTISVDKSKNQFSLKLSSVTAADTAVYYCARLPGYESAFDIWGQGTMVTVSSGGGGSGGGGSGGGGSEIVLTQSPGTLSLSPGERATLSCRASQSVSSSYLAWYQQKPGQAPRLLIYGASSRATGIPDRFSGSGSGTDFTLTISRLEPEDFAVYYCQQAGLFPYTFGGGTKVEIK

SEQ ID NO: 28 - protein, 246 aa, Artificial
  M971 scFv amino acid sequence
QVQLQQSGPGLVKPSQTLSLTCAISGDSVSSNSAAWNWIRQSPSRGLEWLGRTYYRSKWYNDYAVSVKSRITINPDTSKNQFSLQLNSVTPEDTAVYYCAREVTGDLEDAFDIWGQGTMVTVSSGGGGSGGGGSGGGGSDIQMTQSPSSLSASVGDRVTITCRASQTIWSYLNWYQQRPGKAPNLLIYAASSLQSGVPSRFSGRGSGTDFTLTISSLQAEDFATYYCQQSYSIPQTFGQGTKLEIK

SEQ ID NO: 29 - protein, 18 aa, Artificial
  T2A amino acid sequence
EGRGSLLTCGDVEENPGP

SEQ ID NO: 30 - protein, 21 aa, Artificial
  CD8α signal peptide amino acid sequence
MALPVTALLLPLALLLHAARP

SEQ ID NO: 31 - protein, 83 aa, Artificial
  CD8α hinge region and transmembrane region amino acid sequence
FVPVFLPAKPTTTPAPRPPTPAPTIASQPLSLRPEACRPAAGGAVHTRGLDFACDIYIWAPLAGTCGVLLLSLVITLYCNHRN

SEQ ID NO: 32 - protein, 42 aa, Artificial
  4-1BB costimulatory signaling domain amino acid sequence
KRGRKKLLYIFKQPFMRPVQTTQEEDGCSCRFPEEEEGGCEL

SEQ ID NO: 33 - protein, 112 aa, Artificial
  CD3z intracellular signaling domain amino acid sequence
RVKFSRSADAPAYQQGQNQLYNELNLGRREEYDVLDKRRGRDPEMGGKPRRKNPQEGLYNELQKDKMAEAYSEIGMKGERRRGKGHDGLYQGLSTATKDTYDALHMQALPPR

SEQ ID NO: 34 - protein, 357 aa, Artificial
  tEGFR amino acid sequence
MLLLVTSLLLCELPHPAFLLIPRKVCNGIGIGEFKDSLSINATNIKHFKNCTSISGDLHILPVAFRGDSFTHTPPLDPQELDILKTVKEITGFLLIQAWPENRTDLHAFENLEIIRGRTKQHGQFSLAVVSLNITSLGLRSLKEISDGDVIISGNKNLCYANTINWKKLFGTSGQKTKIISNRGENSCKATGQVCHALCSPEGCWGPEPRDCVSCRNVSRGRECVDKCNLLEGEPREFVENSECIQCHPECLPQAMNITCTGRGPDNCIQCAHYIDGPHCVKTCPAGVMGENNTLVWKYADAGHVCHLCHPNCTYGCTGPGLEGCPTNGPKIPSIATGMVGALLLLLVVALGIGLFM

SEQ ID NO: 35 - protein, 520 aa, Artificial
  Clone 17 CAR amino acid sequence
MALPVTALLLPLALLLHAARPEVQLLESGGGLVQPGGSLRLSCAASGFTFSSYAMSWVRQAPGKGLEWVSAISGSGGSTYYADSVKGRFTISRDNSKNTLYLQMNSLRAEDTAVYYCAKVGISSLHGMDVWGQGTTVTVSSGGGGSGGGGSGGGGSDIQMTQSPSTLSASVGDRVTITCRASQSISSWLAWYQQKPGKAPKLLIYKASSLESGVPSRFSGSGSGTEFTLTISSLQPDDFATYYCQQYERFPWTFGGGTKVEIKFVPVFLPAKPTTTPAPRPPTPAPTIASQPLSLRPEACRPAAGGAVHTRGLDFACDIYIWAPLAGTCGVLLLSLVITLYCNHRNKRGRKKLLYIFKQPFMRPVQTTQEEDGCSCRFPEEEEGGCELRVKFSRSADAPAYQQGQNQLYNELNLGRREEYDVLDKRRGRDPEMGGKPRRKNPQEGLYNELQKDKMAEAYSEIGMKGERRRGKGHDGLYQGLSTATKDTYDALHMQALPPRGSGEGRGSLLTCGDVEENPG

SEQ ID NO: 36 - protein, 517 aa, Artificial
  Clone 28 CAR amino acid sequence
MALPVTALLLPLALLLHAARPQVQLQESGPGLVKPSETLSLTCTVSGGSISSYYWSWIRQPAGKGLEWIGRIYTSGSTNYNPSLKSRVTMSVDTSKNQFSLKLSSVTAADTAVYYCARDLYRDGMDVWGQGTTVTVSSGGGGSGGGGSGGGGSDIQMTQSPSTLSASVGDRVTITCRASQSISSWLAWYQQKPGKAPKLLISDASSLESGVPSRFSGSGSGTEFTLTISSLQPDDFATYYCQQANTYSPTFGGGTKVEIKFVPVFLPAKPTTTPAPRPPTPAPTIASQPLSLRPEACRPAAGGAVHTRGLDFACDIYIWAPLAGTCGVLLLSLVITLYCNHRNKRGRKKLLYIFKQPFMRPVQTTQEEDGCSCRFPEEEEGGCELRVKFSRSADAPAYQQGQNQLYNELNLGRREEYDVLDKRRGRDPEMGGKPRRKNPQEGLYNELQKDKMAEAYSEIGMKGERRRGKGHDGLYQGLSTATKDTYDALHMQALPPRGSGEGRGSLLTCGDVEENPG

SEQ ID NO: 37 - protein, 520 aa, Artificial
  Clone 80 CAR amino acid sequence
MALPVTALLLPLALLLHAARPQVQLQESGPGLVKPSGTLSLTCAVSGGSISSSNWWSWVRQPPGKGLEWIGEIYHSGSTNYNPSLKSRVTISVDKSKNQFSLKLSSVTAADTAVYYCARLPGYESAFDIWGQGTMVTVSSGGGGSGGGGSGGGGSEIVLTQSPGTLSLSPGERATLSCRASQSVSSSYLAWYQQKPGQAPRLLIYGASSRATGIPDRFSGSGSGTDFTLTISRLEPEDFAVYYCQQAGLFPYTFGGGTKVEIKFVPVFLPAKPTTTPAPRPPTPAPTIASQPLSLRPEACRPAAGGAVHTRGLDFACDIYIWAPLAGTCGVLLLSLVITLYCNHRNKRGRKKLLYIFKQPFMRPVQTTQEEDGCSCRFPEEEEGGCELRVKFSRSADAPAYQQGQNQLYNELNLGRREEYDVLDKRRGRDPEMGGKPRRKNPQEGLYNELQKDKMAEAYSEIGMKGERRRGKGHDGLYQGLSTATKDTYDALHMQALPPRGSGEGRGSLLTCGDVEENPG

SEQ ID NO: 38 - DNA, 726 bp, Artificial
  Clone 17 scFv nucleotide sequence
gaggtgcagctgttggagtctgggggaggcttggtacagcctggggggtccctgagactctcctgtgcagcctctggattcacctttagcagctatgccatgagctgggtccgccaggctccagggaaggggctggagtgggtctcagctattagtggtagtggtggtagcacatactacgcagactccgtgaagggccggttcaccatctccagagacaattccaagaacacgctgtatctgcaaatgaacagcctgagagccgaggacacggcggtgtactactgcgccaaggtaggaatatccagcttacacggaatggacgtatggggccagggaacaactgtcaccgtcagctcaggtggcgggggcagcggcggaggcggatccggaggcggagggagtgacatccagatgacccagtctccttccaccctgtctgcatctgtaggagacagagtcaccatcacttgccgggccagtcagagtattagtagctggttggcctggtatcagcagaaaccagggaaagcccctaagctcctgatctataaagcctccagtttggaaagtggggtcccatcaaggttcagcggcagtggatctgggacagaattcactctcaccatcagcagcctgcagcctgatgattttgcaacttattactgccagcagtacgaacgcttcccttggacttttggcggagggaccaaggttgagatcaaa

SEQ ID NO: 39 - DNA, 717 bp, Artificial
  Clone 28 scFv nucleotide sequence
caggtgcagctgcaggagtcgggcccaggactggtgaagccttcggagaccctgtccctcacctgcactgtctctggtggctccatcagtagttactactggagctggatccggcagcccgccgggaagggactggagtggattgggcgtatctataccagtgggagcaccaactacaacccctccctcaagagtcgagtcaccatgtcagtagacacgtccaagaaccagttctccctgaagctgagctctgtgaccgccgcggacacggcggtgtactactgcgccagagacttgtacagagatggaatggacgtatggggccagggaacaactgtcaccgtcagctcaggtggcgggggcagcggcggaggcggatccggaggcggagggagtgacatccagatgacccagtctccttccaccctgtctgcatctgtaggagacagagtcaccatcacttgccgggccagtcagagtattagtagctggttggcctggtatcagcagaaaccagggaaagcccctaagctcctgatctccgatgcctccagtttggaaagtggggtcccatcaaggttcagcggcagtggatctgggacagaattcactctcaccatcagcagcctgcagcctgatgattttgcaacttattactgccagcaggccaatacctactctcctacttttggcggagggaccaaggttgagatcaaa

SEQ ID NO: 40 - DNA, 726 bp, Artificial
  Clone 80 scFv nucleotide sequence
caggtgcagctgcaggagtcgggcccaggactggtgaagccttcggggaccctgtccctcacctgcgctgtctctggtggctccatcagcagtagtaactggtggagttgggtccgccagcccccagggaaggggctggagtggattggggaaatctatcatagtgggagcaccaactacaacccgtccctcaagagtcgagtcaccatatcagtagacaagtccaagaaccagttctccctgaagctgagctctgtgaccgccgcggacacggcggtgtactactgcgccagacttcctggatacgagtcagctttcgacatatggggtcagggtacaatggtcaccgtcagctcaggtggcgggggcagcggcggaggcggatccggaggcggagggagtgaaattgtgttgacgcagtctccaggcaccctgtctttgtctccaggggaaagagccaccctctcctgcagggccagtcagagtgttagcagcagctacttagcctggtaccagcagaaacctggccaggctcccaggctcctcatctatggtgcatccagcagggccactggcatcccagacaggttcagtggcagtgggtctgggacagacttcactctcaccatcagcagactggagcctgaagattttgcagtgtattactgtcagcaggccggactcttcccttacacttttggcggagggaccaaggttgagatcaaa

SEQ ID NO: 41 - DNA, 738 bp, Artificial
  M971 scFv nucleotide sequence
caggtgcagctccagcagagcggccccggcctggtaaagcccagccaaaccctctccctgacctgcgctatcagcggcgattccgtgagcagcaacagcgccgcctggaattggatccgtcagagccccagcaggggcctggagtggctggggcggacctattaccggagtaagtggtacaacgactacgccgtaagcgtgaagagccgcatcaccattaatcctgacaccagcaagaaccagttcagtctgcagctgaacagcgtgactcccgaggacaccgccgtgtactactgcgcccgcgaggtgactggagacctggaagacgccttcgacatctggggccagggcacaatggtgaccgtcagcagcggtggcgggggcagcggcggaggcggatccggaggcggagggagtgacatacagatgacccagagccctagcagcctctctgccagcgtgggagaccgggtgaccatcacctgccgcgccagtcagaccatctggtcttatctgaactggtaccagcaacggcccggcaaggcccctaacctgttgatctacgccgccagcagtctccagagcggcgttccatctcgcttcagcggccgcggcagcggcacagacttcaccctgaccatcagcagcctgcaggccgaggacttcgccacctactactgccagcagagctacagcatcccccagactttcggacagggcaccaagttggagatcaaa

SEQ ID NO: 42 - DNA, 2276 bp, Artificial
  Nucleotide sequence  of CAR portion in PXL0662
gccgccaccatggccctgcctgtgacagctctgctcctccctctggccctgctgctccatgccgccagacccgagacgtgagaattaatacgactcactatagagggactggtgaaatgcagttcaaggtttacacctataaaagagagagccgctatcgcctgtttgtggatgtacagagtgatattattgacacgcccgggcgacggatggtgatccccctggccagtgcacgtctgctgtcagataaagtctcccgtgaactttacccggtggtgcatatcggggatgaaagctggcgcatgatgaccacccagatggtcagtgtgccggtctccgtcatcggagaagaagtggctgatctcagccaccgcgaaaatgacatcaaaaacgccattaatctgatgttctggggaatataacgtctcttcgtgcccgtgttcctgcccgccaaacctaccaccacccctgcccctagacctcccaccccagccccaacaatcgccagccagcctctgtctctgcggcccgaagcctgtagacctgctgccggcggagccgtgcacaccagaggcctggacttcgcctgcgacatctacatctgggcccctctggccggcacctgtggcgtgctgctgctgagcctggtgatcaccctgtactgcaaccaccggaacaaacggggcagaaagaaactcctgtatatattcaaacaaccatttatgagaccagtacaaactactcaagaggaagatggctgtagctgccgatttccagaagaagaagaaggaggatgtgaactgagagtgaagttcagcagatccgccgacgcccctgcctaccagcagggacagaaccagctgtacaacgagctgaacctgggcagacgggaagagtacgacgtgctggacaagcggagaggccgggaccccgagatgggcggaaagcccagacggaagaacccccaggaaggcctgtataacgaactgcagaaagacaagatggccgaggcctacagcgagatcggcatgaagggcgagcggaggcgcggcaagggccacgatggcctgtaccagggcctgagcaccgccaccaaggacacctacgacgccctgcacatgcaggccctgccccccagaggatccggagagggaaggggcagcttattaacatgtggcgatgtggaagagaaccccggtcccatgctgctgctcgtgacctctttactgttatgtgagctgccccaccccgcttttttactgatccctcgtaaggtgtgtaacggaatcggcattggcgagttcaaggactctttaagcatcaacgccacaaacatcaagcacttcaagaattgtacctccatcagcggcgatttacacattctccccgtggcttttcgtggcgattccttcacccacaccccccctctggacccccaagagctggacattttaaaaaccgtgaaggagatcaccggctttctgctgatccaagcttggcccgagaatcgtaccgacctccacgccttcgagaatttagagattattcgtggaaggaccaagcagcacggccagttctctttagccgtcgtgtctttaaacattaccagcctcggtttaaggtctttaaaggagattagcgacggcgacgtgatcatctccggcaacaagaacctctgctacgccaacaccatcaactggaagaagctgttcggaaccagcggccaaaagaccaagatcatcagcaatcgtggagagaactcttgtaaggccactggtcaagtttgccacgccctctgtagccccgaaggatgttggggccccgagcctagggactgtgttagctgcagaaacgtgagcagaggcagagagtgtgtggacaaatgcaatttactggaaggagagcctagggagttcgtggagaacagcgaatgtatccagtgccaccccgagtgtttacctcaagccatgaacatcacttgtaccggaaggggccccgataactgcatccaatgcgcccactacatcgacggaccccactgcgtgaaaacttgtcccgccggagtgatgggagagaataacactttagtgtggaagtacgccgacgctggccacgtctgccatctgtgccaccccaactgtacctacggctgcactggtcccggtttagagggatgtcctaccaacggccccaagatcccctccatcgccaccggaatggtgggcgctctgttattactgctggtggtggctctgggcatcggtttattcatgtga

SEQ ID NO: 43 - DNA, 2637 bp, Artificial
  Clone 17 CAR nucleotide sequence
atggccctgcctgtgacagctctgctcctccctctggccctgctgctccatgccgccagacccgaggtgcagctgttggagtctgggggaggcttggtacagcctggggggtccctgagactctcctgtgcagcctctggattcacctttagcagctatgccatgagctgggtccgccaggctccagggaaggggctggagtgggtctcagctattagtggtagtggtggtagcacatactacgcagactccgtgaagggccggttcaccatctccagagacaattccaagaacacgctgtatctgcaaatgaacagcctgagagccgaggacacggcggtgtactactgcgccaaggtaggaatatccagcttacacggaatggacgtatggggccagggaacaactgtcaccgtcagctcaggtggcgggggcagcggcggaggcggatccggaggcggagggagtgacatccagatgacccagtctccttccaccctgtctgcatctgtaggagacagagtcaccatcacttgccgggccagtcagagtattagtagctggttggcctggtatcagcagaaaccagggaaagcccctaagctcctgatctataaagcctccagtttggaaagtggggtcccatcaaggttcagcggcagtggatctgggacagaattcactctcaccatcagcagcctgcagcctgatgattttgcaacttattactgccagcagtacgaacgcttcccttggacttttggcggagggaccaaggttgagatcaaattcgtgcccgtgttcctgcccgccaaacctactactacccctgcacctaggcctcccaccccagccccaacaatcgccagccagcctctgtctctgcggcccgaagcctgtagacctgctgccggcggagccgtgcacaccagaggcctggacttcgcctgcgacatctacatctgggcccctctggccggcacctgtggcgtgctgctgctgagcctggtgatcaccctgtactgcaaccaccggaacaaacggggcagaaagaaactcctgtatatattcaaacaaccatttatgagaccagtacaaactactcaagaggaagatggctgtagctgccgatttccagaagaagaagaaggaggatgtgaactgagagtgaagttcagcagatccgccgacgcccctgcctaccagcagggacagaaccagctgtacaacgagctgaacctgggcagacgggaagagtacgacgtgctggacaagcggagaggccgggaccccgagatgggcggaaagcccagacggaagaacccccaggaaggcctgtataacgaactgcagaaagacaagatggccgaggcctacagcgagatcggcatgaagggcgagcggaggcgcggcaagggccacgatggcctgtaccagggcctgagcaccgccaccaaggacacctacgacgccctgcacatgcaggccctgccccccagaggatccggagagggaaggggcagcttattaacatgtggcgatgtggaagagaaccccggtcccatgctgctgctcgtgacctctttactgttatgtgagctgccccaccccgcttttttactgatccctcgtaaggtgtgtaacggaatcggcattggcgagttcaaggactctttaagcatcaacgccacaaacatcaagcacttcaagaattgtacctccatcagcggcgatttacacattctccccgtggcttttcgtggcgattccttcacccacaccccccctctggacccccaagagctggacattttaaaaaccgtgaaggagatcaccggctttctgctgatccaagcttggcccgagaatcgtaccgacctccacgccttcgagaatttagagattattcgtggaaggaccaagcagcacggccagttctctttagccgtcgtgtctttaaacattaccagcctcggtttaaggtctttaaaggagattagcgacggcgacgtgatcatctccggcaacaagaacctctgctacgccaacaccatcaactggaagaagctgttcggaaccagcggccaaaagaccaagatcatcagcaatcgtggagagaactcttgtaaggccactggtcaagtttgccacgccctctgtagccccgaaggatgttggggccccgagcctagggactgtgttagctgcagaaacgtgagcagaggcagagagtgtgtggacaaatgcaatttactggaaggagagcctagggagttcgtggagaacagcgaatgtatccagtgccaccccgagtgtttacctcaagccatgaacatcacttgtaccggaaggggccccgataactgcatccaatgcgcccactacatcgacggaccccactgcgtgaaaacttgtcccgccggagtgatgggagagaataacactttagtgtggaagtacgccgacgctggccacgtctgccatctgtgccaccccaactgtacctacggctgcactggtcccggtttagagggatgtcctaccaacggccccaagatcccctccatcgccaccggaatggtgggcgctctgttattactgctggtggtggctctgggcatcggtttattcatgtga

SEQ ID NO: 44 - DNA, 2628 bp, Artificial
  Clone 28 CAR nucleotide sequence
atggccctgcctgtgacagctctgctcctccctctggccctgctgctccatgccgccagaccccaggtgcagctgcaggagtcgggcccaggactggtgaagccttcggagaccctgtccctcacctgcactgtctctggtggctccatcagtagttactactggagctggatccggcagcccgccgggaagggactggagtggattgggcgtatctataccagtgggagcaccaactacaacccctccctcaagagtcgagtcaccatgtcagtagacacgtccaagaaccagttctccctgaagctgagctctgtgaccgccgcggacacggcggtgtactactgcgccagagacttgtacagagatggaatggacgtatggggccagggaacaactgtcaccgtcagctcaggtggcgggggcagcggcggaggcggatccggaggcggagggagtgacatccagatgacccagtctccttccaccctgtctgcatctgtaggagacagagtcaccatcacttgccgggccagtcagagtattagtagctggttggcctggtatcagcagaaaccagggaaagcccctaagctcctgatctccgatgcctccagtttggaaagtggggtcccatcaaggttcagcggcagtggatctgggacagaattcactctcaccatcagcagcctgcagcctgatgattttgcaacttattactgccagcaggccaatacctactctcctacttttggcggagggaccaaggttgagatcaaattcgtgcccgtgttcctgcccgccaaacccactactacaccagcacccagacctcccaccccagccccaacaatcgccagccagcctctgtctctgcggcccgaagcctgtagacctgctgccggcggagccgtgcacaccagaggcctggacttcgcctgcgacatctacatctgggcccctctggccggcacctgtggcgtgctgctgctgagcctggtgatcaccctgtactgcaaccaccggaacaaacggggcagaaagaaactcctgtatatattcaaacaaccatttatgagaccagtacaaactactcaagaggaagatggctgtagctgccgatttccagaagaagaagaaggaggatgtgaactgagagtgaagttcagcagatccgccgacgcccctgcctaccagcagggacagaaccagctgtacaacgagctgaacctgggcagacgggaagagtacgacgtgctggacaagcggagaggccgggaccccgagatgggcggaaagcccagacggaagaacccccaggaaggcctgtataacgaactgcagaaagacaagatggccgaggcctacagcgagatcggcatgaagggcgagcggaggcgcggcaagggccacgatggcctgtaccagggcctgagcaccgccaccaaggacacctacgacgccctgcacatgcaggccctgccccccagaggatccggagagggaaggggcagcttattaacatgtggcgatgtggaagagaaccccggtcccatgctgctgctcgtgacctctttactgttatgtgagctgccccaccccgcttttttactgatccctcgtaaggtgtgtaacggaatcggcattggcgagttcaaggactctttaagcatcaacgccacaaacatcaagcacttcaagaattgtacctccatcagcggcgatttacacattctccccgtggcttttcgtggcgattccttcacccacaccccccctctggacccccaagagctggacattttaaaaaccgtgaaggagatcaccggctttctgctgatccaagcttggcccgagaatcgtaccgacctccacgccttcgagaatttagagattattcgtggaaggaccaagcagcacggccagttctctttagccgtcgtgtctttaaacattaccagcctcggtttaaggtctttaaaggagattagcgacggcgacgtgatcatctccggcaacaagaacctctgctacgccaacaccatcaactggaagaagctgttcggaaccagcggccaaaagaccaagatcatcagcaatcgtggagagaactcttgtaaggccactggtcaagtttgccacgccctctgtagccccgaaggatgttggggccccgagcctagggactgtgttagctgcagaaacgtgagcagaggcagagagtgtgtggacaaatgcaatttactggaaggagagcctagggagttcgtggagaacagcgaatgtatccagtgccaccccgagtgtttacctcaagccatgaacatcacttgtaccggaaggggccccgataactgcatccaatgcgcccactacatcgacggaccccactgcgtgaaaacttgtcccgccggagtgatgggagagaataacactttagtgtggaagtacgccgacgctggccacgtctgccatctgtgccaccccaactgtacctacggctgcactggtcccggtttagagggatgtcctaccaacggccccaagatcccctccatcgccaccggaatggtgggcgctctgttattactgctggtggtggctctgggcatcggtttattcatgtga

SEQ ID NO: 45 - DNA, 2637 bp, Artificial
  Clone 80 CAR nucleotide sequence
atggccctgcctgtgacagctctgctcctccctctggccctgctgctccatgccgccagaccccaggtgcagctgcaggagtcgggcccaggactggtgaagccttcggggaccctgtccctcacctgcgctgtctctggtggctccatcagcagtagtaactggtggagttgggtccgccagcccccagggaaggggctggagtggattggggaaatctatcatagtgggagcaccaactacaacccgtccctcaagagtcgagtcaccatatcagtagacaagtccaagaaccagttctccctgaagctgagctctgtgaccgccgcggacacggcggtgtactactgcgccagacttcctggatacgagtcagctttcgacatatggggtcagggtacaatggtcaccgtcagctcaggtggcgggggcagcggcggaggcggatccggaggcggagggagtgaaattgtgttgacgcagtctccaggcaccctgtctttgtctccaggggaaagagccaccctctcctgcagggccagtcagagtgttagcagcagctacttagcctggtaccagcagaaacctggccaggctcccaggctcctcatctatggtgcatccagcagggccactggcatcccagacaggttcagtggcagtgggtctgggacagacttcactctcaccatcagcagactggagcctgaagattttgcagtgtattactgtcagcaggccggactcttcccttacacttttggcggagggaccaaggttgagatcaaattcgtgcccgtgttcctgcccgccaaaccaactactactcctgccccaaggccacccaccccagccccaacaatcgccagccagcctctgtctctgcggcccgaagcctgtagacctgctgccggcggagccgtgcacaccagaggcctggacttcgcctgcgacatctacatctgggcccctctggccggcacctgtggcgtgctgctgctgagcctggtgatcaccctgtactgcaaccaccggaacaaacggggcagaaagaaactcctgtatatattcaaacaaccatttatgagaccagtacaaactactcaagaggaagatggctgtagctgccgatttccagaagaagaagaaggaggatgtgaactgagagtgaagttcagcagatccgccgacgcccctgcctaccagcagggacagaaccagctgtacaacgagctgaacctgggcagacgggaagagtacgacgtgctggacaagcggagaggccgggaccccgagatgggcggaaagcccagacggaagaacccccaggaaggcctgtataacgaactgcagaaagacaagatggccgaggcctacagcgagatcggcatgaagggcgagcggaggcgcggcaagggccacgatggcctgtaccagggcctgagcaccgccaccaaggacacctacgacgccctgcacatgcaggccctgccccccagaggatccggagagggaaggggcagcttattaacatgtggcgatgtggaagagaaccccggtcccatgctgctgctcgtgacctctttactgttatgtgagctgccccaccccgcttttttactgatccctcgtaaggtgtgtaacggaatcggcattggcgagttcaaggactctttaagcatcaacgccacaaacatcaagcacttcaagaattgtacctccatcagcggcgatttacacattctccccgtggcttttcgtggcgattccttcacccacaccccccctctggacccccaagagctggacattttaaaaaccgtgaaggagatcaccggctttctgctgatccaagcttggcccgagaatcgtaccgacctccacgccttcgagaatttagagattattcgtggaaggaccaagcagcacggccagttctctttagccgtcgtgtctttaaacattaccagcctcggtttaaggtctttaaaggagattagcgacggcgacgtgatcatctccggcaacaagaacctctgctacgccaacaccatcaactggaagaagctgttcggaaccagcggccaaaagaccaagatcatcagcaatcgtggagagaactcttgtaaggccactggtcaagtttgccacgccctctgtagccccgaaggatgttggggccccgagcctagggactgtgttagctgcagaaacgtgagcagaggcagagagtgtgtggacaaatgcaatttactggaaggagagcctagggagttcgtggagaacagcgaatgtatccagtgccaccccgagtgtttacctcaagccatgaacatcacttgtaccggaaggggccccgataactgcatccaatgcgcccactacatcgacggaccccactgcgtgaaaacttgtcccgccggagtgatgggagagaataacactttagtgtggaagtacgccgacgctggccacgtctgccatctgtgccaccccaactgtacctacggctgcactggtcccggtttagagggatgtcctaccaacggccccaagatcccctccatcgccaccggaatggtgggcgctctgttattactgctggtggtggctctgggcatcggtttattcatgtga